European Patent Specification EP 3 406 721 B1, published October 4, 2023. Title: Method for screening a nucleic acid aptamar. Applicant: The University of Tokyo. The sequence listing filed with the application follows.

SEQUENCE LISTING (33 sequences)

SEQ ID NO: 1 - DNA, 70 bp, Artificial Sequence
  DNA Library
agcagcacagaggtcagatggtttgggtggttaggtgttgacctgggatgcctatgcgtgctaccgtgaa

SEQ ID NO: 2 - DNA, 70 bp, Artificial Sequence
  DNA Library
agcagcacagaggtcagatggagtcgggtggctattgggtatggaccgtgcctatgcgtgctaccgtgaa

SEQ ID NO: 3 - DNA, 70 bp, Artificial Sequence
  DNA Library
agcagcacagaggtcagatggatggtgtaggttgggagaggctcagtgcccctatgcgtgctaccgtgaa

SEQ ID NO: 4 - DNA, 70 bp, Artificial Sequence
  DNA Library
agcagcacagaggtcagatgttggtggggtggctttgggtatttacttggcctatgcgtgctaccgtgaa

SEQ ID NO: 5 - DNA, 70 bp, Artificial Sequence
  DNA Library
agcagcacagaggtcagatggtggatttgggtggattggtatgaactgaccctatgcgtgctaccgtgaa

SEQ ID NO: 6 - DNA, 70 bp, Artificial Sequence
  DNA Library
agcagcacagaggtcagatggttgggtagggttggataggggcaagtagacctatgcgtgctaccgtgaa

SEQ ID NO: 7 - DNA, 70 bp, Artificial Sequence
  DNA Library
agcagcacagaggtcagatggtgtactattatggtgtggttggtatggttcctatgcgtgctaccgtgaa

SEQ ID NO: 8 - DNA, 70 bp, Artificial Sequence
  DNA Library
agcagcacagaggtcagatgggttgggtggtgtgggtagtgatccctgtgcctatgcgtgctaccgtgaa

SEQ ID NO: 9 - DNA, 70 bp, Artificial Sequence
  DNA Library
agcagcacagaggtcagatgtggattggttggattgggggtgtgactgtgcctatgcgtgctaccgtgaa

SEQ ID NO: 10 - DNA, 70 bp, Artificial Sequence
  DNA Library
agcagcacagaggtcagatgtcgggttggattggttggcttaaactatgtcctatgcgtgctaccgtgaa

SEQ ID NO: 11 - DNA, 71 bp, Artificial Sequence
  DNA Library
agcagcacagaggtcagatgtctggttggtgtggttgggagttttttgatccctatgcgtgctaccgtgaa

SEQ ID NO: 12 - DNA, 70 bp, Artificial Sequence; identical to SEQ ID NO: 3
  DNA Library

SEQ ID NO: 13 - DNA, 70 bp, Artificial Sequence; identical to SEQ ID NO: 1
  DNA Library

SEQ ID NO: 14 - DNA, 69 bp, Artificial Sequence
  DNA Library
agcagcacagaggtcagatggatggtgtaggttgggagaggctcagtgccctatgcgtgctaccgtgaa

SEQ ID NO: 15 - DNA, 70 bp, Artificial Sequence
  DNA Library
agcagcacagaggtcagatgttagggttgggagggtggctgactaatgtacctatgcgtgctaccgtgaa

SEQ ID NO: 16 - DNA, 70 bp, Artificial Sequence; identical to SEQ ID NO: 2
  DNA Library

SEQ ID NO: 17 - DNA, 70 bp, Artificial Sequence
  DNA Library
agcagcacagaggtcagatggggttggattgggtggcggtgtgaactatgcctatgcgtgctaccgtgaa

SEQ ID NO: 18 - DNA, 70 bp, Artificial Sequence
  DNA Library
agcagcacagaggtcagatggttggttatggtggttttagtgggactcgacctatgcgtgctaccgtgaa

SEQ ID NO: 19 - DNA, 69 bp, Artificial Sequence
  DNA Library
agcagcacagaggtcagatgataggatgggtgggtgggttcgtcagttacctatgcgtgctaccgtgaa

SEQ ID NO: 20 - DNA, 70 bp, Artificial Sequence
  DNA Library
agcagcacagaggtcagatgtgggtccggggttgggggggtggccgggtccctatgcgtgctaccgtgaa

SEQ ID NO: 21 - DNA, 70 bp, Artificial Sequence
  DNA Library
agcagcacagaggtcagatggggtggggtggattggttggcgttcctggacctatgcgtgctaccgtgaa

SEQ ID NO: 22 - DNA, 70 bp, Artificial Sequence
  DNA Library
agcagcacagaggtcagatgaagagggtggagtggttggcttcacaatggcctatgcgtgctaccgtgaa

SEQ ID NO: 23 - DNA, 70 bp, Artificial Sequence; identical to SEQ ID NO: 18
  DNA Library

SEQ ID NO: 24 - DNA, 70 bp, Artificial Sequence
  DNA Library
agcagcacagaggtcagatgggggtggatgtggtattttagtggcgatctcctatgcgtgctaccgtgaa

SEQ ID NO: 25 - DNA, 70 bp, Artificial Sequence
  DNA Library
agcagcacagaggtcagatgaagggggtgggggtcgggtggcctcacgatcctatgcgtgctaccgtgaa

SEQ ID NO: 26 - DNA, 70 bp, Artificial Sequence
  DNA Library
agcagcacagaggtcagatgggatggattggttggcgtctgataatggtgcctatgcgtgctaccgtgaa

SEQ ID NO: 27 - DNA, 70 bp, Artificial Sequence; identical to SEQ ID NO: 1
  DNA Library

SEQ ID NO: 28 - DNA, 70 bp, Artificial Sequence; identical to SEQ ID NO: 3
  DNA Library

SEQ ID NO: 29 - DNA, 70 bp, Artificial Sequence; identical to SEQ ID NO: 4
  DNA Library

SEQ ID NO: 30 - DNA, 70 bp, Artificial Sequence
  DNA Library
agcagcacagaggtcagatgggggatggttagggtggcttaatattgacccctatgcgtgctaccgtgaa

SEQ ID NO: 31 - DNA, 69 bp, Artificial Sequence
  DNA Library
agcagcacagaggtcagatgacggggatgggggggtggaggaggcctgtcctatgcgtgctaccgtgaa

SEQ ID NO: 32 - DNA, 20 bp, Artificial Sequence
  primer
agcagcacagaggtcagatg

SEQ ID NO: 33 - DNA, 20 bp, Artificial Sequence
  primer
ttcacggtagcacgcatagg